European Patent Specification EP 4 168 033 B1, published February 25, 2026. Title: ADMINISTRATION OF CEBP-BETA ANTAGONIST AND METHODS OF USE. Applicant: SAPIENCE THERAPEUTICS, INC. The sequence listing filed with the application follows.

SEQUENCE LISTING (4 sequences)

SEQ ID NO: 1 - protein, 22 aa, Artificial Sequence
  Description of Artificial Sequence: Synthetic peptide
  MOD_RES (1)..(22): D-amino acid
VAEAREELERLEARLGQARGEL

SEQ ID NO: 2 - protein, 38 aa, Artificial Sequence
  Description of Artificial Sequence: Synthetic polypeptide
  MOD_RES (1)..(38): D-amino acid
VAEAREELERLEARLGQARGELKKWKMRRNQFWLKLQR

SEQ ID NO: 3 - protein, 22 aa, Unknown
  Description of Unknown: ATF5 bZIP domain peptide
LEGECQGLEARNRELKERAESV

SEQ ID NO: 4 - protein, 22 aa, Unknown
  Description of Unknown: bZIP domain peptide
LEGRAQGLRAELRELEERAEAV